European Patent Application EP 4 218 827 A1, published August 2, 2023. Title: Composition for Preventing or Treating Dmentia Comprising Peptide Nucleic Acid Complex. Applicant: SEASUN THERAPEUTICS, Inc. The sequence listing filed with the application follows.

SEQUENCE LISTING (14 sequences)

SEQ ID NO: 1 - DNA, 15 bp, Artificial Sequence
  Bioactive nucleic acid
acgtgcattatctga

SEQ ID NO: 2 - DNA, 15 bp, Artificial Sequence
  Bioactive nucleic acid
tcgatcattagcgtg

SEQ ID NO: 3 - DNA, 15 bp, Artificial Sequence
  Bioactive nucleic acid
acgtgcattatctga

SEQ ID NO: 4 - DNA, 15 bp, Artificial Sequence
  Bioactive nucleic acid
acctctacgcaatcc

SEQ ID NO: 5 - DNA, 15 bp, Artificial Sequence
  Carrier peptide nucleic acid
tggagatgcgttagg

SEQ ID NO: 6 - DNA, 15 bp, Artificial Sequence
  Carrier peptide nucleic acid
agctagtaatcgcac

SEQ ID NO: 7 - DNA, 15 bp, Artificial Sequence
  Carrier peptide nucleic acid
cacgctaatgatcga

SEQ ID NO: 8 - DNA, 5 bp, Artificial Sequence
  Carrier peptide nucleic acid
cgcac

SEQ ID NO: 9 - DNA, 5 bp, Artificial Sequence
  Carrier peptide nucleic acid
cacgc

SEQ ID NO: 10 - DNA, 15 bp, Artificial Sequence
  Carrier peptide nucleic acid
tgcacgtaatagact

SEQ ID NO: 11 - DNA, 15 bp, Artificial Sequence
  Carrier peptide nucleic acid
tcagataatgcacgt

SEQ ID NO: 12 - DNA, 5 bp, Artificial Sequence
  Carrier peptide nucleic acid
agact

SEQ ID NO: 13 - DNA, 6 bp, Artificial Sequence
  Carrier peptide nucleic acid
tcagac

SEQ ID NO: 14 - DNA, 15 bp, Artificial Sequence
  Carrier peptide nucleic acid
tgcacgtaatagact